European Patent Specification EP 3 801 499 B1, published February 28, 2024. Title: Inhibitors of SARM1. Applicant: DisArm Therapeutics, Inc. The sequence listing filed with the application follows.

SEQUENCE LISTING (1 sequence)

SEQ ID NO: 1 - DNA, 10329 bp, Artificial Sequence
  Chemically synthesized oligonucleotide
gtcgacggatcgggagatctcccgatcccctatggtgcactctcagtacaatctgctctgatgccgcatagttaagccagtatctgctccctgcttgtgtgttggaggtcgctgagtagtgcgcgagcaaaatttaagctacaacaaggcaaggcttgaccgacaattgcatgaagaatctgcttagggttaggcgttttgcgctgcttcgcgatgtacgggccagatatacgcgttgacattgattattgactagttattaatagtaatcaattacggggtcattagttcatagcccatatatggagttccgcgttacataacttacggtaaatggcccgcctggctgaccgcccaacgacccccgcccattgacgtcaataatgacgtatgttcccatagtaacgccaatagggactttccattgacgtcaatgggtggagtatttacggtaaactgcccacttggcagtacatcaagtgtatcatatgccaagtacgccccctattgacgtcaatgacggtaaatggcccgcctggcattatgcccagtacatgaccttatgggactttcctacttggcagtacatctacgtattagtcatcgctattaccatggtgatgcggttttggcagtacatcaatgggcgtggatagcggtttgactcacggggatttccaagtctccaccccattgacgtcaatgggagtttgttttggcaccaaaatcaacgggactttccaaaatgtcgtaacaactccgccccattgacgcaaatgggcggtaggcgtgtacggtgggaggtctatataagcagcgcgttttgcctgtactgggtctctctggttagaccagatctgagcctgggagctctctggctaactagggaacccactgcttaagcctcaataaagcttgccttgagtgcttcaagtagtgtgtgcccgtctgttgtgtgactctggtaactagagatccctcagacccttttagtcagtgtggaaaatctctagcagtggcgcccgaacagggacttgaaagcgaaagggaaaccagaggagctctctcgacgcaggactcggcttgctgaagcgcgcacggcaagaggcgaggggcggcgactggtgagtacgccaaaaattttgactagcggaggctagaaggagagagatgggtgcgagagcgtcagtattaagcgggggagaattagatcgcgatgggaaaaaattcggttaaggccagggggaaagaaaaaatataaattaaaacatatagtatgggcaagcagggagctagaacgattcgcagttaatcctggcctgttagaaacatcagaaggctgtagacaaatactgggacagctacaaccatcccttcagacaggatcagaagaacttagatcattatataatacagtagcaaccctctattgtgtgcatcaaaggatagagataaaagacaccaaggaagctttagacaagatagaggaagagcaaaacaaaagtaagaccaccgcacagcaagcggccgctgatcttcagacctggaggaggagatatgagggacaattggagaagtgaattatataaatataaagtagtaaaaattgaaccattaggagtagcacccaccaaggcaaagagaagagtggtgcagagagaaaaaagagcagtgggaataggagctttgttccttgggttcttgggagcagcaggaagcactatgggcgcagcgtcaatgacgctgacggtacaggccagacaattattgtctggtatagtgcagcagcagaacaatttgctgagggctattgaggcgcaacagcatctgttgcaactcacagtctggggcatcaagcagctccaggcaagaatcctggctgtggaaagatacctaaaggatcaacagctcctggggatttggggttgctctggaaaactcatttgcaccactgctgtgccttggaatgctagttggagtaataaatctctggaacagatttggaatcacacgacctggatggagtgggacagagaaattaacaattacacaagcttaatacactccttaattgaagaatcgcaaaaccagcaagaaaagaatgaacaagaattattggaattagataaatgggcaagtttgtggaattggtttaacataacaaattggctgtggtatataaaattattcataatgatagtaggaggcttggtaggtttaagaatagtttttgctgtactttctatagtgaatagagttaggcagggatattcaccattatcgtttcagacccacctcccaaccccgaggggacccgacaggcccgaaggaatagaagaagaaggtggagagagagacagagacagatccattcgattagtgaacggatcggcactgcgtgcgccaattctgcagacaaatggcagtattcatccacaattttaaaagaaaaggggggattggggggtacagtgcaggggaaagaatagtagacataatagcaacagacatacaaactaaagaattacaaaaacaaattacaaaaattcaaaattttcgggtttattacagggacagcagagatccagtttggttaattaagggtgcagcggcctccgcgccgggttttggcgcctcccgcgggcgcccccctcctcacggcgagcgctgccacgtcagacgaagggcgcaggagcgttcctgatccttccgcccggacgctcaggacagcggcccgctgctcataagactcggccttagaaccccagtatcagcagaaggacattttaggacgggacttgggtgactctagggcactggttttctttccagagagcggaacaggcgaggaaaagtagtcccttctcggcgattctgcggagggatctccgtggggcggtgaacgccgatgattatataaggacgcgccgggtgtggcacagctagttccgtcgcagccgggatttgggtcgcggttcttgtttgtggatcgctgtgatcgtcacttggtgagttgcgggctgctgggctggccggggctttcgtggccgccgggccgctcggtgggacggaagcgtgtggagagaccgccaagggctgtagtctgggtccgcgagcaaggttgccctgaactgggggttggggggagcgcacaaaatggcggctgttcccgagtcttgaatggaagacgcttgtaaggcgggctgtgaggtcgttgaaacaaggtggggggcatggtgggcggcaagaacccaaggtcttgaggccttcgctaatgcgggaaagctcttattcgggtgagatgggctggggcaccatctggggaccctgacgtgaagtttgtcactgactggagaactcgggtttgtcgtctggttgcgggggcggcagttatgcggtgccgttgggcagtgcacccgtacctttgggagcgcgcgcctcgtcgtgtcgtgacgtcacccgttctgttggcttataatgcagggtggggccacctgccggtaggtgtgcggtaggcttttctccgtcgcaggacgcagggttcgggcctagggtaggctctcctgaatcgacaggcgccggacctctggtgaggggagggataagtgaggcgtcagtttctttggtcggttttatgtacctatcttcttaagtagctgaagctccggttttgaactatgcgctcggggttggcgagtgtgttttgtgaagttttttaggcaccttttgaaatgtaatcatttgggtcaatatgtaattttcagtgttagactagtaaagcttctgcaggtcgactctagaaaattgtccgctaaattctggccgtttttggcttttttgttagacgaagcttgggctgcaggtcgactctagaggatccggatccgccaccatgtcagcttggagccacccacaattcgaaaaaggcggtggctcaggcggtggctcaggtggctcagcttggagccacccacaattcgaaaaaggcggtggctcatctggcggaggtggcggtggctcatctggcggaggtgctagcgtgcccagctggaaggaggccgaggttcagacgtggctgcagcagatcggtttctccaagtactgcgagagcttccgggagcagcaggtggatggcgacctgcttctgcggctcacggaggaggaactccagaccgacctgggcatgaaatcgggcatcacccgcaagaggttctttagggagctcacggagctcaagaccttcgccaactattctacgtgcgaccgcagcaacctggcggactggctgggcagcctggacccgcgcttccgccagtacacctacggcctggtcagctgcggcctggaccgctccctgctgcaccgcgtgtctgagcagcagctgctggaagactgcggcatccacctgggcgtgcaccgcgcccgcatcctcacggcggccagagaaatgctacactccccgctgccctgtactggtggcaaacccagtggggacactccagatgtcttcatcagctaccgccggaactcaggttcccagctggccagtctcctgaaggtgcacctgcagctgcatggcttcagtgtcttcattgatgtggagaagctggaagcaggcaagttcgaggacaaactcatccagagtgtcatgggtgcccgcaactttgtgttggtgctatcacctggagcactggacaagtgcatgcaagaccatgactgcaaggattgggtgcataaggagattgtgactgctttaagctgcggcaagaacattgtgcccatcattgatggcttcgagtggcctgagccccaggtcctgcctgaggacatgcaggctgtgcttactttcaacggtatcaagtggtcccacgaataccaggaggccaccattgagaagatcatccgcttcctgcagggccgctcctcccgggactcatctgcaggctctgacaccagtttggagggtgctgcacccatgggtccaacctaaactctagaattcgatatcaagcttatcgataatcaacctctggattacaaaatttgtgaaagattgactggtattcttaactatgttgctccttttacgctatgtggatacgctgctttaatgcctttgtatcatgctattgcttcccgtatggctttcattttctcctccttgtataaatcctggttgctgtctctttatgaggagttgtggcccgttgtcaggcaacgtggcgtggtgtgcactgtgtttgctgacgcaacccccactggttggggcattgccaccacctgtcagctcctttccgggactttcgctttccccctccctattgccacggcggaactcatcgccgcctgccttgcccgctgctggacaggggctcggctgttgggcactgacaattccgtggtgttgtcggggaaatcatcgtcctttccttggctgctcgcctgtgttgccacctggattctgcgcgggacgtccttctgctacgtcccttcggccctcaatccagcggaccttccttcccgcggcctgctgccggctctgcggcctcttccgcgtcttcgccttcgccctcagacgagtcggatctccctttgggccgcctccccgcatcgataccgtcgacctcgagacctagaaaaacatggagcaatcacaagtagcaatacagcagctaccaatgctgattgtgcctggctagaagcacaagaggaggaggaggtgggttttccagtcacacctcaggtacctttaagaccaatgacttacaaggcagctgtagatcttagccactttttaaaagaaaaggggggactggaagggctaattcactcccaacgaagacaagatatccttgatctgtggatctaccacacacaaggctacttccctgattggcagaactacacaccagggccagggatcagatatccactgacctttggatggtgctacaagctagtaccagttgagcaagagaaggtagaagaagccaatgaaggagagaacacccgcttgttacaccctgtgagcctgcatgggatggatgacccggagagagaagtattagagtggaggtttgacagccgcctagcatttcatcacatggcccgagagctgcatccggactgtactgggtctctctggttagaccagatctgagcctgggagctctctggctaactagggaacccactgcttaagcctcaataaagcttgccttgagtgcttcaagtagtgtgtgcccgtctgttgtgtgactctggtaactagagatccctcagacccttttagtcagtgtggaaaatctctagcagggcccgtttaaacccgctgatcagcctcgactgtgccttctagttgccagccatctgttgtttgcccctcccccgtgccttccttgaccctggaaggtgccactcccactgtcctttcctaataaaatgaggaaattgcatcgcattgtctgagtaggtgtcattctattctggggggtggggtggggcaggacagcaagggggaggattgggaagacaatagcaggcatgctggggatgcggtgggctctatggcttctgaggcggaaagaaccagctggggctctagggggtatccccacgcgccctgtagcggcgcattaagcgcggcgggtgtggtggttacgcgcagcgtgaccgctacacttgccagcgccctagcgcccgctcctttcgctttcttcccttcctttctcgccacgttcgccggctttccccgtcaagctctaaatcgggggctccctttagggttccgatttagtgctttacggcacctcgaccccaaaaaacttgattagggtgatggttcacgtagtgggccatcgccctgatagacggtttttcgccctttgacgttggagtccacgttctttaatagtggactcttgttccaaactggaacaacactcaaccctatctcggtctattcttttgatttataagggattttgccgatttcggcctattggttaaaaaatgagctgatttaacaaaaatttaacgcgaattaattctgtggaatgtgtgtcagttagggtgtggaaagtccccaggctccccagcaggcagaagtatgcaaagcatgcatctcaattagtcagcaaccaggtgtggaaagtccccaggctccccagcaggcagaagtatgcaaagcatgcatctcaattagtcagcaaccatagtcccgcccctaactccgcccatcccgcccctaactccgcccagttccgcccattctccgccccatggctgactaattttttttatttatgcagaggccgaggccgcctctgcctctgagctattccagaagtagtgaggaggcttttttggaggcctaggcttttgcaaaaagctcccgggagcttgtatatccattttcggatctgatcagcacgtgttgacaattaatcatcggcatagtatatcggcatagtataatacgacaaggtgaggaactaaaccatggccaagttgaccagtgccgttccggtgctcaccgcgcgcgacgtcgccggagcggtcgagttctggaccgaccggctcgggttctcccgggacttcgtggaggacgacttcgccggtgtggtccgggacgacgtgaccctgttcatcagcgcggtccaggaccaggtggtgccggacaacaccctggcctgggtgtgggtgcgcggcctggacgagctgtacgccgagtggtcggaggtcgtgtccacgaacttccgggacgcctccgggccggccatgaccgagatcggcgagcagccgtgggggcgggagttcgccctgcgcgacccggccggcaactgcgtgcacttcgtggccgaggagcaggactgacacgtgctacgagatttcgattccaccgccgccttctatgaaaggttgggcttcggaatcgttttccgggacgccggctggatgatcctccagcgcggggatctcatgctggagttcttcgcccaccccaacttgtttattgcagcttataatggttacaaataaagcaatagcatcacaaatttcacaaataaagcatttttttcactgcattctagttgtggtttgtccaaactcatcaatgtatcttatcatgtctgtataccgtcgacctctagctagagcttggcgtaatcatggtcatagctgtttcctgtgtgaaattgttatccgctcacaattccacacaacatacgagccggaagcataaagtgtaaagcctggggtgcctaatgagtgagctaactcacattaattgcgttgcgctcactgcccgctttccagtcgggaaacctgtcgtgccagctgcattaatgaatcggccaacgcgcggggagaggcggtttgcgtattgggcgctcttccgcttcctcgctcactgactcgctgcgctcggtcgttcggctgcggcgagcggtatcagctcactcaaaggcggtaatacggttatccacagaatcaggggataacgcaggaaagaacatgtgagcaaaaggccagcaaaaggccaggaaccgtaaaaaggccgcgttgctggcgtttttccataggctccgcccccctgacgagcatcacaaaaatcgacgctcaagtcagaggtggcgaaacccgacaggactataaagataccaggcgtttccccctggaagctccctcgtgcgctctcctgttccgaccctgccgcttaccggatacctgtccgcctttctcccttcgggaagcgtggcgctttctcatagctcacgctgtaggtatctcagttcggtgtaggtcgttcgctccaagctgggctgtgtgcacgaaccccccgttcagcccgaccgctgcgccttatccggtaactatcgtcttgagtccaacccggtaagacacgacttatcgccactggcagcagccactggtaacaggattagcagagcgaggtatgtaggcggtgctacagagttcttgaagtggtggcctaactacggctacactagaagaacagtatttggtatctgcgctctgctgaagccagttaccttcggaaaaagagttggtagctcttgatccggcaaacaaaccaccgctggtagcggtggtttttttgtttgcaagcagcagattacgcgcagaaaaaaaggatctcaagaagatcctttgatcttttctacggggtctgacgctcagtggaacgaaaactcacgttaagggattttggtcatgagattatcaaaaaggatcttcacctagatccttttaaattaaaaatgaagttttaaatcaatctaaagtatatatgagtaaacttggtctgacagttaccaatgcttaatcagtgaggcacctatctcagcgatctgtctatttcgttcatccatagttgcctgactccccgtcgtgtagataactacgatacgggagggcttaccatctggccccagtgctgcaatgataccgcgagacccacgctcaccggctccagatttatcagcaataaaccagccagccggaagggccgagcgcagaagtggtcctgcaactttatccgcctccatccagtctattaattgttgccgggaagctagagtaagtagttcgccagttaatagtttgcgcaacgttgttgccattgctacaggcatcgtggtgtcacgctcgtcgtttggtatggcttcattcagctccggttcccaacgatcaaggcgagttacatgatcccccatgttgtgcaaaaaagcggttagctccttcggtcctccgatcgttgtcagaagtaagttggccgcagtgttatcactcatggttatggcagcactgcataattctcttactgtcatgccatccgtaagatgcttttctgtgactggtgagtactcaaccaagtcattctgagaatagtgtatgcggcgaccgagttgctcttgcccggcgtcaatacgggataataccgcgccacatagcagaactttaaaagtgctcatcattggaaaacgttcttcggggcgaaaactctcaaggatcttaccgctgttgagatccagttcgatgtaacccactcgtgcacccaactgatcttcagcatcttttactttcaccagcgtttctgggtgagcaaaaacaggaaggcaaaatgccgcaaaaaagggaataagggcgacacggaaatgttgaatactcatactcttcctttttcaatattattgaagcatttatcagggttattgtctcatgagcggatacatatttgaatgtatttagaaaaataaacaaataggggttccgcgcacatttccccgaaaagtgccacctgac